European Patent Application EP 4 682 160 A1, published January 21, 2026. Title: Protein and Vaccine Against Infection by SARS-CoV-2 Omicron Variant XBB and Subvariants Thereof. Applicant: WestVac Biopharma Co., Ltd. Application CN. The sequence listing filed with the application follows.

SEQUENCE LISTING (28 sequences)

SEQ ID NO: 1 - protein, 324 aa, synthetic construct
VQPTESIVRFPNITNLCPFDEVFNATRFASVYAWNRKRISNCVADYSVLYNFAPFFAFKCYGVSPTKLNDLCFTNVYADSFVIRGNEVSQIAPGQTGNIADYNYKLPDDFTGCVIAWNSNKLDSKVGGNYNYRYRLFRKSNLKPFERDISTEIYQAGNKPCNGVAGVNCYFPLQSYGFRPTYGVGHQPYRVVVLSFELLHAPATVCGPKKSTNLVKNKSVNFNFNGLYENQKLIANQFNSAIGKIQDSLSSTASALGKLQDVVNQNAQALNTLVKQLKNHTSPDVDLGDISGINASVVNIQKEIDRLNEVAKNLNESLIDLQEL

SEQ ID NO: 2 - protein, 324 aa, synthetic construct
VQPTESIVRFPNITNLCPFDEVFNATRFASVYAWNRKRISNCVADYSVLYNSASFSAFKCYGVSPTKLNDLCFTNVYADSFVIRGNEVSQIAPGQTGNIADYNYKLPDDFTGCVIAWNSNKLDSKVGGNYNYRYRLFRKSNLKPFERDISTEIYQAGNKPCNGVAGVNCYFPLQSYGFRPTYGVGHQPYRVVVLSFELLHAPATVCGPKKSTNLVKNKSVNFNFNGLYENQKLIANQFNSAIGKIQDSLSSTASALGKLQDVVNQNAQALNTLVKQLKNHTSPDVDLGDISGINASVVNIQKEIDRLNEVAKNLNESLIDLQEL

SEQ ID NO: 3 - protein, 226 aa, synthetic construct
VQPTESIVRFPNITNLCPFHEVFNATTFASVYAWNRKRISNCVADYSVIYNFAPFFAFKCYGVSPTKLNDLCFTNVYADSFVIRGNEVSQIAPGQTGNIADYNYKLPDDFTGCVIAWNSNKLDSKPSGNYNYLYRLFRKSKLKPFERDISTEIYQAGNKPCNGVAGPNCYSPLQSYGFRPTYGVGHQPYRVVVLSFELLHAPATVCGPKKSTNLVKNKCVNFNFNG

SEQ ID NO: 4 - protein, 226 aa, synthetic construct
VQPTESIVRFPNITNLCPFHEVFNATTFASVYAWNRKRISNCVADYSVIYNSASFSAFKCYGVSPTKLNDLCFTNVYADSFVIRGNEVSQIAPGQTGNIADYNYKLPDDFTGCVIAWNSNKLDSKPSGNYNYLYRLFRKSKLKPFERDISTEIYQAGNKPCNGVAGPNCYSPLQSYGFRPTYGVGHQPYRVVVLSFELLHAPATVCGPKKSTNLVKNKCVNFNFNG

SEQ ID NO: 5 - protein, 324 aa, synthetic construct
VQPTESIVRFPNITNLCPFHEVFNATTFASVYAWNRKRISNCVADYSVIYNFAPFFAFKCYGVSPTKLNDLCFTNVYADSFVIRGNEVSQIAPGQTGNIADYNYKLPDDFTGCVIAWNSNKLDSKPSGNYNYLYRLFRKSKLKPFERDISTEIYQAGNKPCNGVAGPNCYSPLQSYGFRPTYGVGHQPYRVVVLSFELLHAPATVCGPKKSTNLVKNKSVNFNFNGLYENQKLIANQFNSAIGKIQDSLSSTASALGKLQDVVNQNAQALNTLVKQLKNHTSPDVDLGDISGINASVVNIQKEIDRLNEVAKNLNESLIDLQEL

SEQ ID NO: 6 - protein, 324 aa, synthetic construct
VQPTESIVRFPNITNLCPFHEVFNATTFASVYAWNRKRISNCVADYSVIYNSASFSAFKCYGVSPTKLNDLCFTNVYADSFVIRGNEVSQIAPGQTGNIADYNYKLPDDFTGCVIAWNSNKLDSKPSGNYNYLYRLFRKSKLKPFERDISTEIYQAGNKPCNGVAGPNCYSPLQSYGFRPTYGVGHQPYRVVVLSFELLHAPATVCGPKKSTNLVKNKSVNFNFNGLYENQKLIANQFNSAIGKIQDSLSSTASALGKLQDVVNQNAQALNTLVKQLKNHTSPDVDLGDISGINASVVNIQKEIDRLNEVAKNLNESLIDLQEL

SEQ ID NO: 7 - protein, 1254 aa, synthetic construct
VNLITRTQSYTNSFTRGVYYPDKVFRSSVLHSTQDLFLPFFSNVTWFHAIHVSGTNGTKRFDNPALPFNDGVYFASTEKSNIIRGWIFGTTLDSKTQSLLIVNNATNVVIKVCEFQFCNDPFLDVYQKNNKSWMESEFRVYSSANNCTFEYVSQPFLMDLEGKEGNFKNLREFVFKNIDGYFKIYSKHTPINLERDLPQGFSALEPLVDLPIGINITRFQTLLALHRSYLTPVDSSSGWTAGAAAYYVGYLQPRTFLLKYNENGTITDAVDCALDPLSETKCTLKSFTVEKGIYQTSNFRVQPTESIVRFPNITNLCPFHEVFNATTFASVYAWNRKRISNCVADYSVIYNFAPFFAFKCYGVSPTKLNDLCFTNVYADSFVIRGNEVSQIAPGQTGNIADYNYKLPDDFTGCVIAWNSNKLDSKPSGNYNYLYRLFRKSKLKPFERDISTEIYQAGNKPCNGVAGPNCYSPLQSYGFRPTYGVGHQPYRVVVLSFELLHAPATVCGPKKSTNLVKNKCVNFNFNGLTGTGVLTESNKKFLPFQQFGRDIADTTDAVRDPQTLEILDITPCSFGGVSVITPGTNTSNQVAVLYQGVNCTEVPVAIHADQLTPTWRVYSTGSNVFQTRAGCLIGAEYVNNSYECDIPIGAGICASYQTQTKSHRRARSVASQSIIAYTMSLGAENSVAYSNNSIAIPTNFTISVTTEILPVSMTKTSVDCTMYICGDSTECSNLLLQYGSFCTQLKRALTGIAVEQDKNTQEVFAQVKQIYKTPPIKYFGGFNFSQILPDPSKPSKRSFIEDLLFNKVTLADAGFIKQYGDCLGDIAARDLICAQKFNGLTVLPPLLTDEMIAQYTSALLAGTITSGWTFGAGAALQIPFAMQMAYRFNGIGVTQNVLYENQKLIANQFNSAIGKIQDSLSSTASALGKLQDVVNHNAQALNTLVKQLSSKFGAISSVLNDILSRLDKVEAEVQIDRLITGRLQSLQTYVTQQLIRAAEIRASANLAATKMSECVLGQSKRVDFCGKGYHLMSFPQSAPHGVVFLHVTYVPAQEKNFTTAPAICHDGKAHFPREGVFVSNGTHWFVTQRNFYEPQIITTDNTFVSGNCDVVIGIVNNTVYDPLQPELDSFKEELDKYFKNHTSPDVDLGDISGINASVVNIQKEIDRLNEVAKNLNESLIDLQELGKYEQYIKWPWYIWLGFIAGLIAIVMVTIMLCCMTSCCSCLKGCCSCGSCCKFDEDDSEPVLKGVKLHYT

SEQ ID NO: 8 - protein, 492 aa, synthetic construct
MLLVNQSHQGFNKEHTSKMVSAIVLYVLLAAAAHSAFAADSIHIKDSDDLKNRLAEAGDKLVVIDFMATWCGPCKMIGPKLDEMANEMSDSIVVLKVDVDECEDIATEYNINSMPTFVFVKNSKKIEEFSGANVDKLRNTIIKLKLAGSGSGHMHHHHHHSSGDDDDKVQPTESIVRFPNITNLCPFDEVFNATRFASVYAWNRKRISNCVADYSVLYNFAPFFAFKCYGVSPTKLNDLCFTNVYADSFVIRGNEVSQIAPGQTGNIADYNYKLPDDFTGCVIAWNSNKLDSKVGGNYNYRYRLFRKSNLKPFERDISTEIYQAGNKPCNGVAGVNCYFPLQSYGFRPTYGVGHQPYRVVVLSFELLHAPATVCGPKKSTNLVKNKSVNFNFNGLYENQKLIANQFNSAIGKIQDSLSSTASALGKLQDVVNQNAQALNTLVKQLKNHTSPDVDLGDISGINASVVNIQKEIDRLNEVAKNLNESLIDLQEL

SEQ ID NO: 9 - DNA, 1479 bp, synthetic construct
  source 1..1479: mol_type = other DNA
atgctgctggtgaaccagagccaccagggtttcaacaaggaacacactagcaagatggtgtctgctatcgtcctctacgtgctgctcgccgccgctgctcactcagctttcgccgctgactctatccacatcaaggactccgacgacctcaagaaccgtttggccgaagccggcgacaagctggtcgttatcgacttcatggctacctggtgtggcccttgcaagatgatcggacctaagctggacgaaatggctaacgagatgagcgacagcatcgtcgttctgaaggtggacgtcgacgaatgtgaggacatcgccactgagtacaacatcaacagcatgcctaccttcgttttcgtgaagaactctaagaagatcgaggagttctctggtgccaacgtggacaagctccgtaacaccatcatcaagctcaagctggccggcagcggtagcggtcacatgcaccaccaccaccaccattcaagcggcgacgacgacgacaaggtgcagccaaccgaatcaatcgtccgcttcccaaacatcactaacctgtgcccattcgacgaggtgttcaacgccacccgtttcgcctctgtctacgcttggaaccgcaagcgcatctccaactgtgtcgccgactacagcgtgctgtacaacttcgctcctttcttcgcattcaagtgttacggagtgtcccctaccaagctcaacgatttgtgcttcacaaacgtgtacgctgacagcttcgtgatccgtggtaacgaggtttctcaaatcgcccctggtcagacaggtaacatcgctgactacaactacaagctcccagacgacttcactggctgtgttatcgcttggaactcaaacaagctggactctaaggtgggtggtaactacaactaccggtaccgtctgttccgcaagagcaacctcaagccattcgaacgtgacatcagcacagagatctaccaagccggtaacaagccctgcaacggcgttgccggagtcaactgctacttccccctccagtcctacggattccgcccaacctacggcgtgggtcaccagccataccgcgtggttgtgctgagcttcgaactgctgcacgcccccgctaccgtgtgtggccctaagaagagcactaacctcgttaagaacaagtccgtgaacttcaacttcaacggtctctacgaaaaccagaagctgatcgctaaccagttcaactccgccatcggcaagatccaggactccctgtcctccacagcttccgctctgggcaagctgcaggacgttgtgaaccaaaacgctcaggccctgaacacactggtgaagcaactgaagaaccacaccagccccgacgttgacctgggtgacatcagcggtatcaacgctagcgtggtgaacatccagaaggagatcgacaggctgaacgaagtggctaagaacttgaacgagagcctcatcgacctgcaggaactgtaa

SEQ ID NO: 10 - protein, 492 aa, synthetic construct
MLLVNQSHQGFNKEHTSKMVSAIVLYVLLAAAAHSAFAADSIHIKDSDDLKNRLAEAGDKLVVIDFMATWCGPCKMIGPKLDEMANEMSDSIVVLKVDVDECEDIATEYNINSMPTFVFVKNSKKIEEFSGANVDKLRNTIIKLKLAGSGSGHMHHHHHHSSGDDDDKVQPTESIVRFPNITNLCPFDEVFNATRFASVYAWNRKRISNCVADYSVLYNSASFSAFKCYGVSPTKLNDLCFTNVYADSFVIRGNEVSQIAPGQTGNIADYNYKLPDDFTGCVIAWNSNKLDSKVGGNYNYRYRLFRKSNLKPFERDISTEIYQAGNKPCNGVAGVNCYFPLQSYGFRPTYGVGHQPYRVVVLSFELLHAPATVCGPKKSTNLVKNKSVNFNFNGLYENQKLIANQFNSAIGKIQDSLSSTASALGKLQDVVNQNAQALNTLVKQLKNHTSPDVDLGDISGINASVVNIQKEIDRLNEVAKNLNESLIDLQEL

SEQ ID NO: 11 - DNA, 1479 bp, synthetic construct
  source 1..1479: mol_type = other DNA
atgctgctggtgaaccagagccaccagggtttcaacaaggaacacactagcaagatggtgtctgctatcgtcctctacgtgctgctcgccgccgctgctcactcagctttcgccgctgactctatccacatcaaggactccgacgacctcaagaaccgtttggccgaagccggcgacaagctggtcgttatcgacttcatggctacctggtgtggcccttgcaagatgatcggacctaagctggacgaaatggctaacgagatgagcgacagcatcgtcgttctgaaggtggacgtcgacgaatgtgaggacatcgccactgagtacaacatcaacagcatgcctaccttcgttttcgtgaagaactctaagaagatcgaggagttctctggtgccaacgtggacaagctccgtaacaccatcatcaagctcaagctggccggcagcggtagcggtcacatgcaccaccaccaccaccattcaagcggcgacgacgacgacaaggtgcagccaaccgaatcaatcgtccgcttcccaaacatcactaacctgtgcccattcgacgaggtgttcaacgccacccgtttcgcctctgtctacgcttggaaccgcaagcgcatctccaactgtgtcgccgactacagcgtgctgtacaactcagcttcattctcagcattcaagtgttacggagtgtcccctaccaagctcaacgatttgtgcttcacaaacgtgtacgctgacagcttcgtgatccgtggtaacgaggtttctcaaatcgcccctggtcagacaggtaacatcgctgactacaactacaagctcccagacgacttcactggctgtgttatcgcttggaactcaaacaagctggactctaaggtgggtggtaactacaactaccggtaccgtctgttccgcaagagcaacctcaagccattcgaacgtgacatcagcacagagatctaccaagccggtaacaagccctgcaacggcgttgccggagtcaactgctacttccccctccagtcctacggattccgcccaacctacggcgtgggtcaccagccataccgcgtggttgtgctgagcttcgaactgctgcacgcccccgctaccgtgtgtggccctaagaagagcactaacctcgttaagaacaagtccgtgaacttcaacttcaacggtctctacgaaaaccagaagctgatcgctaaccagttcaactccgccatcggcaagatccaggactccctgtcctccacagcttccgctctgggcaagctgcaggacgttgtgaaccaaaacgctcaggccctgaacacactggtgaagcaactgaagaaccacaccagccccgacgttgacctgggtgacatcagcggtatcaacgctagcgtggtgaacatccagaaggagatcgacaggctgaacgaagtggctaagaacttgaacgagagcctcatcgacctgcaggaactgtaa

SEQ ID NO: 12 - protein, 394 aa, synthetic construct
MLLVNQSHQGFNKEHTSKMVSAIVLYVLLAAAAHSAFAADSIHIKDSDDLKNRLAEAGDKLVVIDFMATWCGPCKMIGPKLDEMANEMSDCIVVLKVDVDECEDIATEYNINSMPTFVFVKNSKKIEEFSGANVDKLRNTIIKLKLAGSGSGHMHHHHHHSSGDDDDKVQPTESIVRFPNITNLCPFHEVFNATTFASVYAWNRKRISNCVADYSVIYNFAPFFAFKCYGVSPTKLNDLCFTNVYADSFVIRGNEVSQIAPGQTGNIADYNYKLPDDFTGCVIAWNSNKLDSKPSGNYNYLYRLFRKSKLKPFERDISTEIYQAGNKPCNGVAGPNCYSPLQSYGFRPTYGVGHQPYRVVVLSFELLHAPATVCGPKKSTNLVKNKCVNFNFNG

SEQ ID NO: 13 - DNA, 1185 bp, synthetic construct
  source 1..1185: mol_type = other DNA
atgctactagtaaatcagtcacaccaaggtttcaacaaggaacacaccagcaagatggtgagcgctatcgtgctgtacgtcctgctggccgctgctgctcacagcgctttcgctgctgactccatccacatcaaggacagcgacgacctgaagaaccgtctggccgaggccggtgacaagctggtcgtcatcgacttcatggccacttggtgcggtccttgcaagatgatcggccctaagctggacgagatggctaacgagatgtccgactgcatcgtggtcctgaaggtggacgtcgacgagtgcgaggacatcgccaccgaatacaacatcaacagcatgcccaccttcgtgttcgtgaagaacagcaagaagatcgaggaattttccggcgctaacgtcgacaagctgcgtaacaccatcatcaagctgaagctggccggctccggctccggccacatgcatcaccaccaccaccattcctccggtgacgacgacgacaaggtgcagccaaccgaatctatcgtcagattcccaaacatcactaacctgtgccctttccacgaggtgttcaacgctaccactttcgccagcgtctacgcttggaaccgcaagcgtatcagcaactgcgtcgccgactactctgtgatctacaacttcgctcctttcttcgctttcaagtgctacggcgtgtcacctaccaagctgaacgacctgtgcttcactaacgtctacgccgactccttcgtgatccgcggaaacgaagtctctcagatcgctcctggacagaccggaaatatcgctgactacaactacaagctgccagacgacttcactggctgcgtgatcgcttggaactcaaacaagctggactccaagccttctggcaactacaactacctgtacaggctgttcagaaagtcaaagctgaagcctttcgagcgcgacatctcaaccgaaatctaccaggctggtaataagccctgcaacggtgtggctggccctaactgctactctcccctgcagtcctacggtttccgtccaacctacggagtcggtcatcagccttaccgtgtggtcgtgctgagcttcgaactgctccacgctcctgctactgtgtgcggtcccaagaagtctactaacctggtcaaaaacaaatgtgtcaacttcaacttcaacggttaa

SEQ ID NO: 14 - protein, 394 aa, synthetic construct
MLLVNQSHQGFNKEHTSKMVSAIVLYVLLAAAAHSAFAADSIHIKDSDDLKNRLAEAGDKLVVIDFMATWCGPCKMIGPKLDEMANEMSDCIVVLKVDVDECEDIATEYNINSMPTFVFVKNSKKIEEFSGANVDKLRNTIIKLKLAGSGSGHMHHHHHHSSGDDDDKVQPTESIVRFPNITNLCPFHEVFNATTFASVYAWNRKRISNCVADYSVIYNSASFSAFKCYGVSPTKLNDLCFTNVYADSFVIRGNEVSQIAPGQTGNIADYNYKLPDDFTGCVIAWNSNKLDSKPSGNYNYLYRLFRKSKLKPFERDISTEIYQAGNKPCNGVAGPNCYSPLQSYGFRPTYGVGHQPYRVVVLSFELLHAPATVCGPKKSTNLVKNKCVNFNFNG

SEQ ID NO: 15 - DNA, 1185 bp, synthetic construct
  source 1..1185: mol_type = other DNA
atgctactagtaaatcagtcacaccaaggtttcaacaaggaacacaccagcaagatggtgagcgctatcgtgctgtacgtcctgctggccgctgctgctcacagcgctttcgctgctgactccatccacatcaaggacagcgacgacctgaagaaccgtctggccgaggccggtgacaagctggtcgtcatcgacttcatggccacttggtgcggtccttgcaagatgatcggccctaagctggacgagatggctaacgagatgtccgactgcatcgtggtcctgaaggtggacgtcgacgagtgcgaggacatcgccaccgaatacaacatcaacagcatgcccaccttcgtgttcgtgaagaacagcaagaagatcgaggaattttccggcgctaacgtcgacaagctgcgtaacaccatcatcaagctgaagctggccggctccggctccggccacatgcatcaccaccaccaccattcctccggtgacgacgacgacaaggtgcagccaaccgaatctatcgtcagattcccaaacatcactaacctgtgccctttccacgaggtgttcaacgctaccactttcgccagcgtctacgcttggaaccgcaagcgtatcagcaactgcgtcgccgactactctgtgatctacaactccgctagcttctctgctttcaagtgctacggcgtgtcacctaccaagctgaacgacctgtgcttcactaacgtctacgccgactccttcgtgatccgcggaaacgaagtctctcagatcgctcctggacagaccggaaatatcgctgactacaactacaagctgccagacgacttcactggctgcgtgatcgcttggaactcaaacaagctggactccaagccttctggcaactacaactacctgtacaggctgttcagaaagtcaaagctgaagcctttcgagcgcgacatctcaaccgaaatctaccaggctggtaataagccctgcaacggtgtggctggccctaactgctactctcccctgcagtcctacggtttccgtccaacctacggagtcggtcatcagccttaccgtgtggtcgtgctgagcttcgaactgctccacgctcctgctactgtgtgcggtcccaagaagtctactaacctggtcaaaaacaaatgtgtcaacttcaacttcaacggttaa

SEQ ID NO: 16 - protein, 492 aa, synthetic construct
MLLVNQSHQGFNKEHTSKMVSAIVLYVLLAAAAHSAFAADSIHIKDSDDLKNRLAEAGDKLVVIDFMATWCGPCKMIGPKLDEMANEMSDSIVVLKVDVDECEDIATEYNINSMPTFVFVKNSKKIEEFSGANVDKLRNTIIKLKLAGSGSGHMHHHHHHSSGDDDDKVQPTESIVRFPNITNLCPFHEVFNATTFASVYAWNRKRISNCVADYSVIYNFAPFFAFKCYGVSPTKLNDLCFTNVYADSFVIRGNEVSQIAPGQTGNIADYNYKLPDDFTGCVIAWNSNKLDSKPSGNYNYLYRLFRKSKLKPFERDISTEIYQAGNKPCNGVAGPNCYSPLQSYGFRPTYGVGHQPYRVVVLSFELLHAPATVCGPKKSTNLVKNKSVNFNFNGLYENQKLIANQFNSAIGKIQDSLSSTASALGKLQDVVNQNAQALNTLVKQLKNHTSPDVDLGDISGINASVVNIQKEIDRLNEVAKNLNESLIDLQEL

SEQ ID NO: 17 - DNA, 1479 bp, synthetic construct
  source 1..1479: mol_type = other DNA
atgctgctggtgaaccagagccaccagggtttcaacaaggaacacactagcaagatggtgtctgctatcgtcctctacgtgctgctcgccgccgctgctcactcagctttcgccgctgactctatccacatcaaggactccgacgacctcaagaaccgtttggccgaagccggcgacaagctggtcgttatcgacttcatggctacctggtgtggcccttgcaagatgatcggacctaagctggacgaaatggctaacgagatgagcgacagcatcgtcgttctgaaggtggacgtcgacgaatgtgaggacatcgccactgagtacaacatcaacagcatgcctaccttcgttttcgtgaagaactctaagaagatcgaggagttctctggtgccaacgtggacaagctccgtaacaccatcatcaagctcaagctggccggcagcggtagcggtcacatgcaccaccaccaccaccattcaagcggcgacgacgacgacaaggtgcagccaaccgaatcaatcgtccgcttcccaaacatcactaacctgtgcccattccacgaggtgttcaacgccaccactttcgcctctgtctacgcttggaaccgcaagcgcatctccaactgtgtcgccgactacagcgtgatatacaacttcgctcctttcttcgcattcaagtgttacggagtgtcccctaccaagctcaacgatttgtgcttcacaaacgtgtacgctgacagcttcgtgatccgtggtaacgaggtttctcaaatcgcccctggtcagacaggtaacatcgctgactacaactacaagctcccagacgacttcactggctgtgttatcgcttggaactcaaacaagctggactctaagccgtctggtaactacaactacctctaccgtctgttccgcaagagcaagctcaagccattcgaacgtgacatcagcacagagatctaccaagccggtaacaagccctgcaacggcgttgccggacctaactgctactctcccctccagtcctacggattccgcccaacctacggcgtgggtcaccagccataccgcgtggttgtgctgagcttcgaactgctgcacgcccccgctaccgtgtgtggccctaagaagagcactaacctcgttaagaacaagtccgtgaacttcaacttcaacggtctctacgaaaaccagaagctgatcgctaaccagttcaactccgccatcggcaagatccaggactccctgtcctccacagcttccgctctgggcaagctgcaggacgttgtgaaccaaaacgctcaggccctgaacacactggtgaagcaactgaagaaccacaccagccccgacgttgacctgggtgacatcagcggtatcaacgctagcgtggtgaacatccagaaggagatcgacaggctgaacgaagtggctaagaacttgaacgagagcctcatcgacctgcaggaactgtaa

SEQ ID NO: 18 - protein, 492 aa, synthetic construct
MLLVNQSHQGFNKEHTSKMVSAIVLYVLLAAAAHSAFAADSIHIKDSDDLKNRLAEAGDKLVVIDFMATWCGPCKMIGPKLDEMANEMSDSIVVLKVDVDECEDIATEYNINSMPTFVFVKNSKKIEEFSGANVDKLRNTIIKLKLAGSGSGHMHHHHHHSSGDDDDKVQPTESIVRFPNITNLCPFHEVFNATTFASVYAWNRKRISNCVADYSVIYNSASFSAFKCYGVSPTKLNDLCFTNVYADSFVIRGNEVSQIAPGQTGNIADYNYKLPDDFTGCVIAWNSNKLDSKPSGNYNYLYRLFRKSKLKPFERDISTEIYQAGNKPCNGVAGPNCYSPLQSYGFRPTYGVGHQPYRVVVLSFELLHAPATVCGPKKSTNLVKNKSVNFNFNGLYENQKLIANQFNSAIGKIQDSLSSTASALGKLQDVVNQNAQALNTLVKQLKNHTSPDVDLGDISGINASVVNIQKEIDRLNEVAKNLNESLIDLQEL

SEQ ID NO: 19 - DNA, 1479 bp, synthetic construct
  source 1..1479: mol_type = other DNA
atgctgctggtgaaccagagccaccagggtttcaacaaggaacacactagcaagatggtgtctgctatcgtcctctacgtgctgctcgccgccgctgctcactcagctttcgccgctgactctatccacatcaaggactccgacgacctcaagaaccgtttggccgaagccggcgacaagctggtcgttatcgacttcatggctacctggtgtggcccttgcaagatgatcggacctaagctggacgaaatggctaacgagatgagcgacagcatcgtcgttctgaaggtggacgtcgacgaatgtgaggacatcgccactgagtacaacatcaacagcatgcctaccttcgttttcgtgaagaactctaagaagatcgaggagttctctggtgccaacgtggacaagctccgtaacaccatcatcaagctcaagctggccggcagcggtagcggtcacatgcaccaccaccaccaccattcaagcggcgacgacgacgacaaggtgcagccaaccgaatcaatcgtccgcttcccaaacatcactaacctgtgcccattccacgaggtgttcaacgccaccactttcgcctctgtctacgcttggaaccgcaagcgcatctccaactgtgtcgccgactacagcgtgatatacaactccgcttctttctctgcattcaagtgttacggagtgtcccctaccaagctcaacgatttgtgcttcacaaacgtgtacgctgacagcttcgtgatccgtggtaacgaggtttctcaaatcgcccctggtcagacaggtaacatcgctgactacaactacaagctcccagacgacttcactggctgtgttatcgcttggaactcaaacaagctggactctaagccgtctggtaactacaactacctctaccgtctgttccgcaagagcaagctcaagccattcgaacgtgacatcagcacagagatctaccaagccggtaacaagccctgcaacggcgttgccggacctaactgctactctcccctccagtcctacggattccgcccaacctacggcgtgggtcaccagccataccgcgtggttgtgctgagcttcgaactgctgcacgcccccgctaccgtgtgtggccctaagaagagcactaacctcgttaagaacaagtccgtgaacttcaacttcaacggtctctacgaaaaccagaagctgatcgctaaccagttcaactccgccatcggcaagatccaggactccctgtcctccacagcttccgctctgggcaagctgcaggacgttgtgaaccaaaacgctcaggccctgaacacactggtgaagcaactgaagaaccacaccagccccgacgttgacctgggtgacatcagcggtatcaacgctagcgtggtgaacatccagaaggagatcgacaggctgaacgaagtggctaagaacttgaacgagagcctcatcgacctgcaggaactgtaa

SEQ ID NO: 20 - protein, 1269 aa, synthetic construct
MFVFLVLLPLVSSQCVNLITRTQSYTNSFTRGVYYPDKVFRSSVLHSTQDLFLPFFSNVTWFHAIHVSGTNGTKRFDNPALPFNDGVYFASTEKSNIIRGWIFGTTLDSKTQSLLIVNNATNVVIKVCEFQFCNDPFLDVYQKNNKSWMESEFRVYSSANNCTFEYVSQPFLMDLEGKEGNFKNLREFVFKNIDGYFKIYSKHTPINLERDLPQGFSALEPLVDLPIGINITRFQTLLALHRSYLTPVDSSSGWTAGAAAYYVGYLQPRTFLLKYNENGTITDAVDCALDPLSETKCTLKSFTVEKGIYQTSNFRVQPTESIVRFPNITNLCPFHEVFNATTFASVYAWNRKRISNCVADYSVIYNFAPFFAFKCYGVSPTKLNDLCFTNVYADSFVIRGNEVSQIAPGQTGNIADYNYKLPDDFTGCVIAWNSNKLDSKPSGNYNYLYRLFRKSKLKPFERDISTEIYQAGNKPCNGVAGPNCYSPLQSYGFRPTYGVGHQPYRVVVLSFELLHAPATVCGPKKSTNLVKNKCVNFNFNGLTGTGVLTESNKKFLPFQQFGRDIADTTDAVRDPQTLEILDITPCSFGGVSVITPGTNTSNQVAVLYQGVNCTEVPVAIHADQLTPTWRVYSTGSNVFQTRAGCLIGAEYVNNSYECDIPIGAGICASYQTQTKSHRRARSVASQSIIAYTMSLGAENSVAYSNNSIAIPTNFTISVTTEILPVSMTKTSVDCTMYICGDSTECSNLLLQYGSFCTQLKRALTGIAVEQDKNTQEVFAQVKQIYKTPPIKYFGGFNFSQILPDPSKPSKRSFIEDLLFNKVTLADAGFIKQYGDCLGDIAARDLICAQKFNGLTVLPPLLTDEMIAQYTSALLAGTITSGWTFGAGAALQIPFAMQMAYRFNGIGVTQNVLYENQKLIANQFNSAIGKIQDSLSSTASALGKLQDVVNHNAQALNTLVKQLSSKFGAISSVLNDILSRLDKVEAEVQIDRLITGRLQSLQTYVTQQLIRAAEIRASANLAATKMSECVLGQSKRVDFCGKGYHLMSFPQSAPHGVVFLHVTYVPAQEKNFTTAPAICHDGKAHFPREGVFVSNGTHWFVTQRNFYEPQIITTDNTFVSGNCDVVIGIVNNTVYDPLQPELDSFKEELDKYFKNHTSPDVDLGDISGINASVVNIQKEIDRLNEVAKNLNESLIDLQELGKYEQYIKWPWYIWLGFIAGLIAIVMVTIMLCCMTSCCSCLKGCCSCGSCCKFDEDDSEPVLKGVKLHYT

SEQ ID NO: 21 - DNA, 3810 bp, synthetic construct
  source 1..3810: mol_type = other DNA
atgttcgtgttcctggtgctgctgcccctggtgagcagccaatgcgtgaacctgatcacaagaacacagagctacaccaacagcttcacaagaggcgtgtactaccccgacaaggtgttcagaagcagcgtgctgcattccacccaagacctgttcctccccttcttttccaacgtgacctggttccacgccatccacgtgagcggcaccaacggcaccaagagattcgacaaccccgccctgcccttcaacgacggcgtgtacttcgctagcaccgagaagagcaacatcatcagaggctggatcttcggcaccaccctggacagcaagacacagagcctgctgatcgtgaacaatgccaccaacgtggtgatcaaggtgtgcgagtttcagttctgcaacgaccccttcctggacgtgtatcagaagaacaacaagagctggatggagagcgagttcagagtgtacagcagcgctaacaactgcaccttcgagtacgtgagccaacccttcctgatggacctggagggcaaggagggcaacttcaagaacctcagagagttcgtgttcaagaacatcgacggctacttcaagatctacagcaagcacacccccatcaacctggagagagacctgccccaaggcttcagcgccctggagcccctggtggacctgcccatcggcatcaacatcacaagatttcagaccctgctggccctgcacagaagctatctgacacctgtggacagcagcagcggctggacagctggggccgctgcctactacgtgggctacctgcagcctagaaccttcctgctgaagtacaacgagaacggcacaatcaccgatgccgtggattgcgccctggaccccctgagcgagaccaagtgcaccctgaagagcttcaccgtggagaagggcatctatcagacaagcaacttcagagtgcagcccaccgagagcatcgtgagattccccaacatcaccaacctgtgccccttccacgaggtgttcaacgccaccaccttcgctagcgtgtacgcttggaacagaaaaagaatcagcaactgcgtggccgactacagcgtgatctacaacttcgcccccttcttcgccttcaagtgctacggggtgagccccaccaagctgaacgacctgtgcttcaccaacgtgtacgccgacagcttcgtgatcagaggcaacgaggtgagccaaatcgcccctgggcagaccggcaacatcgccgactacaactacaagctgcccgacgacttcaccggctgcgtgatcgcctggaacagcaacaagctggacagcaaacctagcggcaactacaactacctgtacagactgttcagaaagagcaagctgaagcccttcgagagagacatcagcaccgagatctaccaagccggcaacaagccctgcaacggcgtggccggccccaactgctacagccccctgcagagctacggcttcagacccacctacggcgtgggccatcagccctacagagtggtcgtgctgagcttcgagctgctgcacgcccccgccaccgtgtgcggccccaagaagagcaccaacctggtgaagaacaagtgcgtgaacttcaacttcaacggcctcaccggcaccggcgtgctgaccgagagcaacaagaagttcctgccctttcagcagttcggcagagacatcgccgacaccaccgacgccgtgagagaccctcagaccctggagatcctggacatcaccccctgtagcttcggcggcgtgagcgtgatcacccccggcaccaacacaagcaaccaagtggccgtgctgtaccaaggcgtgaactgcaccgaggtgcccgtggccatccacgccgatcagctgacccccacctggagagtctactccaccggcagcaacgtgtttcagacaagagccggctgcctgatcggcgccgagtacgtgaacaacagctacgagtgcgacatccccatcggcgccggcatctgcgctagctatcagacacagaccaagagccacggcagcgctagcagcgtggctagccaaagcatcatcgcctacaccatgagcctgggcgccgagaacagcgtggcctacagcaacaacagcatcgccatccccaccaacttcaccatcagcgtgaccaccgagatcctgcccgtcagcatgaccaagacaagcgtggactgcaccatgtacatctgcggcgacagcaccgagtgcagcaacctgctcctgcagtacggcagcttctgcacacagctgaagagagccctgaccggcatcgccgtggagcaagacaagaacacccaagaggtgttcgcccaagtgaagcagatctacaagaccccccccatcaagtacttcggcggcttcaacttcagccaaatcctccccgacccctccaaacctagcaagagaagcttcatcgaggacctgctgttcaacaaggtgaccctggccgacgccggcttcatcaagcagtacggcgactgcctgggcgatatcgccgctagagacctgatctgcgctcagaagttcaatggcctgaccgtgctgccccccctgctgaccgacgagatgatcgctcagtatacaagcgctctgctcgctggcaccattacaagcgggtggaccttcggcgctggcgctgccctgcagatccccttcgccatgcagatggcctacagattcaacggcatcggcgtgacacagaacgtgctgtacgagaatcagaagctgatcgccaatcagttcaacagcgccatcggcaagatccaagacagcctgagcagcaccgctagcgccctgggcaagctgcaagacgtggtgaaccacaacgcccaagccctgaacaccctggtgaagcagctgagcagcaagttcggcgccatcagcagcgtgctcaacgacatcctgagcagactggacccccccgaggccgaggtgcagatcgatagactgatcaccggcagactgcagagcctgcagacctacgtgacacagcagctgatcagagccgccgagatcagagctagcgccaacctggccgccaccaagatgagcgagtgcgtgctggggcagagcaagagagtggacttctgcggcaagggctaccacctgatgagcttccctcagagcgccccccacggcgtggtgttcctgcacgtgacctacgtgcccgcccaagagaagaacttcaccacagcccccgccatctgccacgacggcaaggcccacttccctagagagggcgtgttcgtgagcaacggcacccactggttcgtgacacagagaaacttctacgagcctcagatcatcaccaccgacaacaccttcgtgagcggcaactgcgacgtggtgatcggcatcgtgaataataccgtgtacgaccccctgcagcccgagctggacagcttcaaggaggagctggacaagtatttcaagaaccatacaagccccgacgtggacctgggcgacatcagcggcatcaacgctagcgtggtgaacattcagaaggaaatcgacagactcaacgaggtggccaagaacctgaacgagagcctgatcgacctgcaagagctgggcaagtacgagcagtacatcaagtggccctggtacatctggctgggcttcatcgccggcctgatcgccatcgtgatggtgaccatcatgctgtgctgcatgacaagctgctgcagctgcctgaagggctgttgcagctgcggcagctgctgcaagttcgacgaggacgacagcgagcccgtgctgaagggcgtgaagctgcactacacctga

SEQ ID NO: 22 - protein, 1268 aa, synthetic construct
MFVFLVLLPLVSSQCVNLITRTQSYTNSFTRGVYYPDKVFRSSVLHSTQDLFLPFFSNVTWFHAISGTNGTKRFDNPVLPFNDGVYFASTEKSNIIRGWIFGTTLDSKTQSLLIVNNATNVVIKVCEFQFCNDPFLDVYYHKNNKSWMESEFRVYSSANNCTFEYVSQPFLMDLEGKQGNFKNLREFVFKNIDGYFKIYSKHTPINLGRDLPQGFSALEPLVDLPIGINITRFQTLLALHRSYLTPGDSSSGWTAGAAAYYVGYLQPRTFLLKYNENGTITDAVDCALDPLSETKCTLKSFTVEKGIYQTSNFRVQPTESIVRFPNITNLCPFDEVFNATRFASVYAWNRKRISNCVADYSVLYNFAPFFAFKCYGVSPTKLNDLCFTNVYADSFVIRGNEVSQIAPGQTGNIADYNYKLPDDFTGCVIAWNSNKLDSKVGGNYNYRYRLFRKSNLKPFERDISTEIYQAGNKPCNGVAGVNCYFPLQSYGFRPTYGVGHQPYRVVVLSFELLHAPATVCGPKKSTNLVKNKCVNFNFNGLTGTGVLTESNKKFLPFQQFGRDIADTTDAVRDPQTLEILDITPCSFGGVSVITPGTNTSNQVAVLYQGVNCTEVPVAIHADQLTPTWRVYSTGSNVFQTRAGCLIGAEYVNNSYECDIPIGAGICASYQTQTKSHRRARSVASQSIIAYTMSLGAENSVAYSNNSIAIPTNFTISVTTEILPVSMTKTSVDCTMYICGDSTECSNLLLQYGSFCTQLKRALTGIAVEQDKNTQEVFAQVKQIYKTPPIKYFGGFNFSQILPDPSKPSKRSFIEDLLFNKVTLADAGFIKQYGDCLGDIAARDLICAQKFNGLTVLPPLLTDEMIAQYTSALLAGTITSGWTFGAGAALQIPFAMQMAYRFNGIGVTQNVLYENQKLIANQFNSAIGKIQDSLSSTASALGKLQDVVNHNAQALNTLVKQLSSKFGAISSVLNDILSRLDPPEAEVQIDRLITGRLQSLQTYVTQQLIRAAEIRASANLAATKMSECVLGQSKRVDFCGKGYHLMSFPQSAPHGVVFLHVTYVPAQEKNFTTAPAICHDGKAHFPREGVFVSNGTHWFVTQRNFYEPQIITTDNTFVSGNCDVVIGIVNNTVYDPLQPELDSFKEELDKYFKNHTSPDVDLGDISGINASVVNIQKEIDRLNEVAKNLNESLIDLQELGKYEQYIKWPWYIWLGFIAGLIAIVMVTIMLCCMTSCCSCLKGCCSCGSCCKFDEDDSEPVLKGVKLHYT

SEQ ID NO: 23 - DNA, 3807 bp, synthetic construct
  source 1..3807: mol_type = other DNA
atgttcgtgttcctggtgctgctgcccctggtgagcagccaatgcgtgaacctgatcacaagaacacagagctacaccaacagcttcacaagaggcgtgtactaccccgacaaggtgttcagaagcagcgtcctgcattccacccaagacctgtttctccccttcttcagcaacgtgacctggttccacgccatcagcggcaccaacggcaccaagagattcgacaaccccgtgctgcccttcaacgacggcgtgtacttcgctagcaccgagaagagcaacatcatcagaggctggatcttcggcaccaccctggacagcaagacacagagcctgctgatcgtgaacaacgccacaaacgtggtgatcaaggtgtgcgagtttcagttctgcaacgaccccttcctggacgtgtactaccacaagaacaacaagagctggatggagagcgagttccgggtgtacagcagcgccaacaactgcaccttcgagtacgtgagccaacccttcctgatggacctggagggcaagcaaggcaacttcaagaacctgagagagttcgtgttcaagaacatcgacggctacttcaagatctacagcaagcacacccccatcaacctgggcagagacctgccccaaggcttcagcgccctggagcccctggtggacctgcccatcggcatcaacatcacaagatttcagacactgctcgccctgcaccggagctacctcacccctggcgacagcagctccggctggaccgctggggctgccgcctactacgtgggctacctgcagcctagaaccttcctgctgaagtacaacgagaacggcaccatcaccgacgctgtggactgtgccctggaccccctgagcgagaccaagtgcaccctgaagagcttcaccgtggagaagggcatctatcagacaagcaacttcagagtgcagcccaccgagagcatcgtgagattccccaacatcaccaacctgtgccccttcgacgaggtgttcaacgccacaagattcgctagcgtgtacgcctggaacagaaagagaatcagcaactgcgtggccgactacagcgtgctgtacaacttcgcccccttcttcgccttcaaatgctacggcgtcagccccaccaagctgaacgacctgtgcttcaccaacgtgtacgccgacagcttcgtgatcagaggcaacgaggtgagccaaatcgcccccgggcagaccggcaacatcgccgactataactacaaactgcccgacgacttcaccggctgcgtgatcgcctggaactccaacaagctggacagcaaagtgggcggcaactacaactacagatacagactgttcagaaagagcaacctgaagcccttcgagagagacatcagcaccgagatctaccaagccggcaacaagccctgcaacggcgtggccggcgtgaactgctacttccccctgcagagctacggcttcagacccacctacggcgtgggccatcagccctacagagtggtcgtgctgagcttcgagctgctgcacgcccctgccacagtgtgcggccccaagaagagcaccaacctggtgaagaacaagtgcgtgaacttcaacttcaacggcctgaccggcaccggcgtgctgaccgagagcaacaagaagttcctgccctttcagcagttcggcagagacatcgccgacaccaccgatgctgtgagagaccctcagaccctggagatcctggacatcaccccttgcagcttcggcggcgtgagcgtgatcacccccggcaccaacacaagcaaccaagtggccgtgctgtaccaaggcgtcaactgcacagaggtgcccgtggccatccacgccgatcagctgacccccacctggagagtgtactccaccggcagcaacgtgtttcagacaagagccggctgcctgatcggcgccgagtacgtgaacaacagctacgagtgcgacatccccatcggcgccggcatctgcgctagctatcagacacagaccaagagccacagaagagctagaagcgtggctagccaaagcatcatcgcctacaccatgagcctgggcgccgagaacagcgtggcctacagcaacaacagcatcgccatccccaccaacttcaccatcagcgtgaccaccgagatcctgcctgtgagcatgaccaagacaagcgtggactgcaccatgtacatctgcggcgacagcaccgagtgcagcaacctgctcctgcagtacggcagcttctgcacacagctgaagagagccctgaccggcatcgccgtggagcaagacaagaacacccaagaggtgttcgcccaagtgaagcagatctacaagaccccccccatcaagtacttcggcggcttcaacttcagccaaatcctgcccgaccctagcaagcctagcaagcggagcttcatcgaggacctgctgttcaacaaggtgaccctggccgacgccggcttcatcaagcagtacggcgactgcctcggcgacatcgctgctagagacctgatctgcgctcagaagttcaacggcctcacagtgctgccccccctgctgaccgacgagatgatcgctcagtacacctccgctctgctggccggcacaattacatccggctggaccttcggcgccggcgccgccctgcaaatccccttcgccatgcagatggcctacagattcaacggcatcggcgtgacacagaacgtgctgtacgagaatcagaagctgatcgccaatcagttcaacagcgccatcggcaagatccaagacagcctgagcagcaccgctagcgccctgggcaagctgcaagacgtggtgaaccacaacgcccaagccctgaacaccctggtgaagcagctgagcagcaagttcggcgccatctcctccgtcctgaacgacatcctgagcagactggacccccccgaggccgaggtgcagattgacagactgattaccggcagactgcagagcctgcagacctacgtgacacagcagctgatcagagccgccgagatcagagctagcgccaacctggccgccaccaagatgagcgagtgcgtgctggggcagagcaagagagtggacttctgcggcaagggctaccacctgatgagcttccctcagagcgccccccacggcgtggtgttcctgcacgtgacctacgtgcccgcccaagagaagaacttcaccaccgctcccgccatctgccacgacggcaaggcccacttccctagagagggcgtgttcgtgagcaacggcacccactggttcgtgacacagagaaacttctacgagcctcagatcatcaccaccgacaacaccttcgtgagcggcaactgcgacgtggtgatcggcatcgtcaacaacaccgtgtacgaccccctgcaacccgagctggacagcttcaaggaggagctggacaagtactttaagaaccacacaagccccgacgtggacctgggggacatctccggcatcaacgctagcgtggtgaacattcagaaggaaattgacagactgaatgaggtggccaagaacctgaacgagagcctgatcgacctgcaagagctgggcaagtacgagcagtacatcaagtggccctggtacatctggctgggcttcatcgccggcctgatcgccatcgtgatggtgaccatcatgctgtgctgcatgacaagctgctgcagctgtctgaagggctgctgctcctgcggcagctgctgcaagttcgacgaggacgacagcgagcccgtgctgaagggcgtgaagctgcactacacctga

SEQ ID NO: 24 - DNA, 21 bp, synthetic construct
  source 1..21: mol_type = other DNA
acacgtcaatgggaagtgaaa

SEQ ID NO: 25 - DNA, 21 bp, synthetic construct
  source 1..21: mol_type = other DNA
gctagacgatccagacatgat

SEQ ID NO: 26 - DNA, 20 bp, synthetic construct
  source 1..20: mol_type = other DNA
gaccccaaaatcagcgaaat

SEQ ID NO: 27 - DNA, 25 bp, synthetic construct
  source 1..25: mol_type = other DNA
tctggttactgcccagttgaatctg

SEQ ID NO: 28 - DNA, 25 bp, synthetic construct
  source 1..25: mol_type = other DNA
acgccgcattacgtttggtgggacc